European Patent Application EP 4 541 892 A1, published April 23, 2025. Title: Transgenic corn event QY2569-42 and detection method thereof. Applicant: Qingdao KingAgroot Seed Science Co., Ltd. The sequence listing filed with the application follows.

SEQUENCE LISTING (40 sequences)

SEQ ID NO: 1 - DNA, 20 bp, Zea mays
  source 1..20: mol_type = genomic DNA
attcgcgcgtagtttaaact

SEQ ID NO: 2 - DNA, 20 bp, Zea mays
  source 1..20: mol_type = genomic DNA
attaaaaacgaccacacgcg

SEQ ID NO: 3 - DNA, 40 bp, Zea mays
  source 1..40: mol_type = genomic DNA
ccatactgtaattcgcgcgtagtttaaactgaaggcggga

SEQ ID NO: 4 - DNA, 40 bp, Zea mays
  source 1..40: mol_type = genomic DNA
aattcagtacattaaaaacgaccacacgcgaacgacacgc

SEQ ID NO: 5 - DNA, 100 bp, Zea mays
  source 1..100: mol_type = genomic DNA
ttaaaacgcaaaacttatgaatgttttaaaccatactgtaattcgcgcgtagtttaaactgaaggcgggaaacgacaatctgatccaagctcaagctgct

SEQ ID NO: 6 - DNA, 100 bp, Zea mays
  source 1..100: mol_type = genomic DNA
tagtgaattcccccgaattaattcggcgttaattcagtacattaaaaacgaccacacgcgaacgacacgcgacaacgcgcggacacttgcaaacgacatg

SEQ ID NO: 7 - DNA, 1269 bp, Zea mays
  source 1..1269: mol_type = genomic DNA
cgaagctacggtcgaggggttagcgcgtttacgttaaacaagtactaattagaacatctaattcaacataattatattaattgatattaatcaaatgtaaattaatactactacttagttttgactaacttactattttaatagttgacaattaagcaagtaacttaatgaatatgagtgattctaagcgagacgaattaacgacgcacgacatgcaaacacgatgtgcgcaacgcgcggacacaaacgacttagcacgcggacaacgcgcgatacgcgcgaacggcacgcggcaatgcgcgcgacacacgcgaacgacacgcgacaacgcgcggacacttgcaaacgacatgcgtgaaacagcaccgcggcacgcgcacggtacgcgcggaccgacatgcgaaactaataaataaatgacaacgtgattacactaaacaattattaatatgtaacatttcagttaaggttaatcatattggtgactaattataaatgcgcgaatcgaattcctaaattagatttttaaattgaaatgtcgttttagtagccactggttaaacaaacgtttaactaaattaaataaaatgtgcaaaaattgggataaatatttctaaattaagattattttaatacgaatctaacgcaacttgaatggatcaaatcggatttaaaacgcaaaacttatgaatgttttaaaccatactgtaattcgcgcgtagtttaaactgaaggcgggaaacgacaatctgatccaagctcaagctgctaagcttattcgggtcaaggcggaagccagcgcgccaccccacgtcagcaaatacggaggcgcggggttgacggcgtcacccggtcctaacggcgaccaacaaaccagccagaagaaattacagtaaaaaaaaagtaaattgcactttgatccaccttttattacctaagtctcaatttggatcacccttaaacctatcttttcaatttgggccgggttgtggtttggactaccatgaacaacttttcgtcatgtctaacttccctttcagcaaacatatgaacaatatatagagaagatcggccgtatactagagctgatgtgtttaaggtcgttgattgcacgagaaaaaaaaatccaaatcgcaacaatagcaaatttatctggttcaaagtgaaaagatatgtttaaaggtagtccaaagtaaaacttatagataataaaatgtggtccaaagcgtaattcactcaaaaaaaatcaacgagacgtgtaccaaacgg

SEQ ID NO: 8 - DNA, 3057 bp, Zea mays
  source 1..3057: mol_type = genomic DNA
ctggcagagggacttcgagctgcccgcgcctccgcgcccggttcgccccgtgacccagatttgatagtttctccataataatgtgtgagtagttcccagataagggaattagggttcctatagggtttcgctcatgtgttgagcatataagaaacccttagtatgtatttgtatttgtaaaatacttctatcaataaaatttctaattcctaaaaccaaaatccagtactaaaatccagatcgggcccactagtgaattcccccgaattaattcggcgttaattcagtacattaaaaacgaccacacgcgaacgacacgcgacaacgcgcggacacttgcaaacgacatgcgtgaaacagcaccgcggcacgcgcacggtacgcgcggaccgacatgcgaaactaataaataaatgacaacgtgattacactaaacaattattaatatgtaacatttcagttaaggttaatcatattggtgactaattataaatgcgcgaatcgaattcctaaattagatttttaaattgaaatgtcgttttagtagccactggttaaacaaacgtttaactaaattaaataaaatgtgcaaaaattgggataaatatttctaaattaagattattttaatacgaatctaacgcaacttgaatggatcaaatcggatttaaaacgcaaaacttatgaatgttttaaaccatactgtaattcgcgcgtcctaatttacagaactgccatcttcttcttcctctcctcatcttcttcctcccatccatggaagagagaggaggggaagggggctgcgcaggggaggacgagaccgggccggccgggggcgggcgcggccgcaccgggcgcgcggggcgcggccacagccgccggggaggggtgcgcgcgggcgtggggcgcgtgagcgcgagcgccaccgccggccaccgccgccgccgccggggagggagaaaggggcgccgtcgaggaggggaaacagaggggggaggggcgccgccaccggggaaggtgaggggagagtgggagaggctctgcacggacgggaaaacgaaaaaaacgaagaaaccctaggtgcaacaatggaggtttctcaccggggaagaagaccctcgccggagccgaggagaaatccgtcgattgccggagattcggggatccaatcgatgaaccgaacgcgctgcgacgaagccttcgacgagacgaacgcagcggtactctcggattctgcagacgatgcacggattgggagtaattgctcgccggagttgtcgccggagttggaaccgccccgaacttcggcgagcaataccgggagctagggattggatttgggggaaacgtttggtgttctggaacgggctcgacgagataaagccggacatgtatatatacctagggtttggacgagacaaaaattcggattttattatttttaaaattcgaaaaagcctagaaatccatattttgtgctcaaaatattatagatactttcaaaaattccagaaaaattcctataaatgttttggcacctaatgaactcaaaaaacataattagaatttctaaaaacatttttaggttccacaaataaatggattttggtttccggaaaatagaaaaatattccgaaaaatatgaaaatttaccgagcgcttctataagatatgttaacatatttgaaacacattttacacttagaaacaccatgcaacgacatgaatgcaacaaccaaagtgcctctagggctcattccactaggtttacgctaatataaaacaaaatgattctccatttttaggaaaaagagaaaggaaagcgaagaactgagagagtaacacctgaatttggtggatattagaaaagaaattttatacccccaaattcagggtgttacaggtgaggagcttaggataatgttatttaactatagggagatgggaattattcctaaggttgagccgatgtaaagtgtggtgccctcgcttgtacatgtgtaaaggcttgtatgttgtgtgcccccgcacacttggctatgcttgcgaaggcgttatgtacttggtctggtgtattttgttatattgtgctggtgcgcatatagtcggtcttggcgcggacagtttggtgtggtcgtttttgcttttgttgtgctagtccggctgcacccttaggcgacttctgcacggatggtcgtcgcggtagacttcggtttttcgcacttgttgtgctagtccggctgcacccttaggcgacttctgcacagatagtcttcgcggtagacttcggtttttcgcacttgttgtgctagtccggctgcacccttaggcgacttctgcacggatagtcttcgcggtagacttcggtttttcgcacttgttgtgctagtccgactgcacccttaggcgacttctgcacggatagtcttcgcggtagacttcggtttttcgcacttgttgtgctagtccgactgcacccttaggcgacttctgcacagatagtcttcgcggtagacttcagtttttcgcacttgttgtgctagtccggctgcacccttaggcgacttctgcacggatagtcttcgcggtagacttaggtttttcgcacttgttgtgctattccggctgcacccttaggcgacttctgcgtggatttgtcgcacgcgagggtggctagcgctgagcctcgcggtgacctcgtattggtcgaatgtcgaagaccgtcgtcgcggtcttttttcgacgcatgtttttgcgggggatttttcatacatatattacatggctccgcctcgttaaaaacctcaccccccgggaggaaaagagtgcgggccagaataagattgtttttgcgaattacaagggcgaatcagccctgatgagtcaaacaaaaaatttgcggaggttgtcgatgttccaggagtgctccaggtcttcgccgtttggcgttgtgagcctgtaagcgctgcgggaagctttcgtcttgactatgaaggggccctcccacctgggctccagcttgcccctggactctgttcgagctgttcggatgagtac

SEQ ID NO: 9 - DNA, 11283 bp, synthetic construct
  source 1..11283: mol_type = other DNA
agtttaaactgaaggcgggaaacgacaatctgatccaagctcaagctgctaagcttattcgggtcaaggcggaagccagcgcgccaccccacgtcagcaaatacggaggcgcggggttgacggcgtcacccggtcctaacggcgaccaacaaaccagccagaagaaattacagtaaaaaaaaagtaaattgcactttgatccaccttttattacctaagtctcaatttggatcacccttaaacctatcttttcaatttgggccgggttgtggtttggactaccatgaacaacttttcgtcatgtctaacttccctttcagcaaacatatgaacaatatatagagaagatcggccgtatactagagctgatgtgtttaaggtcgttgattgcacgagaaaaaaaaatccaaatcgcaacaatagcaaatttatctggttcaaagtgaaaagatatgtttaaaggtagtccaaagtaaaacttatagataataaaatgtggtccaaagcgtaattcactcaaaaaaaatcaacgagacgtgtaccaaacggagacaaacggcatcttctcgaaatttcccaaccgctcgctcgcccgcctcgtcttcccggaaaccgcggtggtttcagcgtggcggattctccaagcagacggagacgtcacggcacgggactcctcccaccacccaaccgccataaataccagccccctcatctcctctcctcgcatcagctccacccccgaaaaatttctccccaatctcgcgaggctctcgtcgtcgaatcgaatcctctcgcgtcctcaaggtacgctgcttctcctctcctcgcttcgtttcgattcgatttcggacgggtgaggttgttttgttgctagatccgattggtggttagggttgtcgatgtgattatcgtgagatgtttaggggttgtagatctgatggttgtgatttgggcacggttggttcgataggtggaatcgtggttaggttttgggattgggatgttggttctgatgattggggggaatttttacggttagatgaattgttggatgattcgattggggaaatcggtgtagatctgttggggaattgtggaactagtcatgcctgagtgattggtgcgatttgtagcgtgttccatcttgtaggccttgttgcgagcatgttcagatctactgttccgctcttgattgagttattggtgccatgggttggtgcaaacacaggctttaatatgttatatctgttttgtgtttgatgtagatctgtagggtagttcttcttagacatggttcaattatgtagcttgtgcgtttcgatttgatttcatatgttcacagattagataatgatgaactcttttaattaattgtcaatggtaaataggaagtcttgtcgctatatctgtcataatgatctcatgttactatctgccagtaatttatgctaagaactatattagaatatcatgttacaatctgtagtaatatcatgttacaatctgtagttcatctatataatctattgtggtaatttctttttactatctgtgtgaagattattgccactagttcattctacttatttctgaagttcaggatacgtgtgctgttactacctatctgaatacatccgtgatgtgcctgttactatctttttgaatacatgtatgttctgttggaatatgtttgctgtttgatccgttgttgtgtccttaatcttgtgctagttcttaccctatctgtttggtgattatttcttgcagaccatggcgcccaccgtgatgatggcctcgtcggccaccgccgtcgcttcgttccaggggctcaagtccaccgccagcctccccgtcgcccgccgctcctccagaagcctcggcaacgtcagcaacggcggaaggatccggtgcatgcaggtgtggccggcctacggcaacaagaagttcgagacgctgtcgtacctgccgccgctgtccaccggcgggcgcatccgctgcatgcaggccatgaacaagaacaacacgaagctctccacccgcggcctgcaaagcttcatcgactacttcaacggcatctacggcttcgcgaccggcatcaaggacatcatgaacatgatcttcaagacggacacgggcggcgacctgacgctcgacgagatcctcaagaaccagcagctcctgaacgacatctcgggcaagctggacggcgtgaacggctccctgaacgacctcatcgcccagggcaacctcaacaccgagctgagcaaggagatcctcaagatcgcgaacgagcagaaccaggtgctgaacgacgtcaacaacaagctcgacgccatcaacaccatgctccgcgtgtacctgcccaagatcacgtccatgctcagcgacgtcatcaagcagaactacgccctgtccctccagatcgagtacctcagcaagcagctgcaggagatctccgacaagctggacatcatcaacgtgaacgtcctcatcaactccaccctgacggagatcaccccggcgtaccagcgcatcaagtatgtgaacgagaagttcgaggagctgacgttcgccaccgagacgtccagcaaggtcaagaaggacggcagccccgccgacatcctggacgagctgaccgagctgacggagctggcgaagtccgtgaccaagaacgacgtcgacggcttcgagttctacctgaacacgttccacgacgtgatggtcggcaacaacctcttcggcaggtcggctctgaagaccgccagcgagctgatcaccaaggagaacgtgaagacgtccggcagcgaagtgggcaacgtctacaacttcctgatcgtcctcacggccctgcaggctcaggcgttcctgaccctgacgacctgccgcaagctcctgggcctcgctgacatcgactacaccagcatcatgaacgagcacctgaacaaggagaaggaggagttcagggtgaacatcctcccgaccctgtccaacacgttcagcaaccccaactacgccaaggtgaagggctccgacgaggacgcgaagatgatcgtggaggctaagcccggccacgccctcatcggcttcgagatctccaacgacagcatcaccgtgctgaaggtctacgaggcgaagctcaagcagaactaccaggtggacaaggactccctgagcgaggtcatctacggcgacatggacaagctcctgtgcccggaccagagcgagcagatctactacaccaacaacatcgtgttccccaacgagtatgtgatcaccaagatcgacttcacgaagaagatgaagaccctccgctacgaggtgaccgccaacttctacgactccagcacgggcgagatcgacctcaacaagaagaaggtcgagtccagcgaggccgagtacaggaccctgagcgcgaacgacgacggcgtgtacatgccgctgggcgtcatctccgagacgttcctcacccccatcaacggcttcggcctgcaggccgacgagaacagccgcctcatcaccctgacgtgcaagtcctacctcagggagctgctgctcgccaccgacctgagcaacaaggagacgaagctcatcgtgccgccctccggcttcatcagcaacatcgtcgagaacggctccatcgaggaggacaacctggagccctggaaggccaacaacaagaacgcctacgtggaccacaccggcggcgtcaacggcacgaaggcgctctacgtgcacaaggacggtggcatcagccagttcatcggcgacaagctgaagccgaagaccgagtatgtgatccagtacacggtcaagggcaagccctccatccacctgaaggacgagaacaccggctacatccactacgaggacacgaacaacaacctcgaggactaccagaccatcaacaagcgcttcaccacgggcacggacctgaagggcgtctacctgatcctcaagtcccagaacggcgacgaggcgtggggcgacaacttcatcatcctcgagatctcgccctcggagaagctgctcagcccggagctgatcaacaccaacaactggacctccacgggcagcacgaacatctccggcaacacgctgaccctctaccagggcggcaggggcatcctcaagcagaacctgcagctcgactccttcagcacctacagggtgtacttctccgtcagcggcgacgcgaacgtgcgcatcaggaactcccgcgaggtcctgttcgagaagaggtacatgtccggcgccaaggacgtgagcgagatgttcaccacgaagttcgagaaggacaacttctacatcgagctgagccagggcaacaacctctacggtggcccgatcgtgcacttctacgacgtctccatcaagtagtgactaggctactgtagctagctgtgcatgtatgtggtgtggttactaaaataattagtgttttccttttgtttggaagcatatgtgtggtgaataaatgatgaactccgatgttcctctctataaatcttgatgattcgctagctatccgtacgtcgttgttctttgatttgatgatgagattgaaaaatggaatgtcatgctaaggagggtgccggtaccgcattccagattgggttcaatcaacaaggtacgagccatatcactttattcaaattggtatcgccaaaaccaagaaggaactcccatcctcaaaggtttgtaaggaagaattctcagtccaaagcctcaacaaggtcagggtacagagtctccaaaccattagccaaaagctacaggagatcaatgaagaatcttcaatcaaagtaaactactgttccagcacatgcatcatggtcagtaagtttcagaaaaagacatccaccgaagacttaaagttagtgggcatctttgaaagtaatcttgtcaacatcgagcagctggcttgtggggaccagacaaaaaaggaatggtgcagaattgttaggcgcacctaccaaaagcatctttgcctttattgcaaagataaagcagattcctctagtacaagtggggaacaaaataacgtggaaaagagctgtcctgacagcccactcactaatgcgtatgacgaacgcagtgacgaccacaaaagaattccctctatataagaaggcattcattcccatttgaaggatcatcagatactcaaccaatccttctaggatctaccgtcttcggtacgcgctcactccgccctctgcctttgttactgccacgtttctctgaatgctctcttgtgtggtgattgctgagagtggtttagctggatctagaattacactctgaaatcgtgttctgcctgtgctgattacttgccgtcctttgtagcagcaaaatatagggacatggtagtacgaaacgaagatagaacctacacagcaatacgagaaatgtgtaatttggtgcttagcggtatttatttaagcacatgttggtgttatagggcacttggattcagaagtttgctgttaatttaggcacaggcttcatactacatgggtcaatagtatagggattcatattataggcgatactataataatttgttcgtctgcagagcttattatttgccaaaattagatattcctattctgtttttgtttgtgtgctgttaaattgttaacgcctgaaggaataaatataaatgacgaaattttgatgtttatctctgctcctttattgtgaccataagtcaagatcagatgcacttgttttaaatattgttgtctgaagaaataagtactgacagtattttgatgcattgatctgcttgtttgttgtaacaaaatttaaaaataaagagtttcctttttgttgctctccttacctcctgatggtatctagtatctaccaactgacactatattgcttctctttacatacgtatcttgctcgatgccttctccctagtgttgaccagtgttactcacatagtctttgctcatttcattgtaatgcagataccaagcggaccatggcgcaagttagcaggatctgcaacggcgtgcagaacccgtcgctcatctccaacctctcgaaatccagtcaacgcaaatcgcccttgtcggtgtccctgaagacgcagcagcacccgcgagcctacccgatctcgtcgtcgtggggcttgaagaagagcgggatgacgctgattggctctgagctccgtcccctcaaggtcatgtcttctgtgtccacggcgtgcatggataataaccctaacatcaatgagtgcattccctacaactgcctgtctaacccagaggtggaggtgctcggcggggagaggattgagacgggctacacgcccatcgacatttccctcagcctgacccagttcctcctgtccgaatttgtcccaggtgccggattcgtgctcggcctcgtcgatatcatttggggtatcttcggaccgagccagtgggacgccttcctcgtgcagattgagcaactcatcaaccagcgcatcgaggaattcgccaggaaccaagcgatttcccgcctcgagggcctctccaacctctaccagatctacgccgaatccttcagggagtgggaagcggatcccaccaacccggccctgagggaggaaatgagaattcagttcaatgacatgaacagcgctttgaccacggcaatcccgctctttgcggtgcagaattaccaggtgccgcttttgtcggtctacgtgcaggccgcgaacctccacctgagcgtcctgagagatgtctcggttttcggtcagcgctggggatttgacgctgcaaccattaattcccgctacaacgacctcacacgcctcatcggcaattacactgaccatgccgtgaggtggtataacaccggcctcgagagggtctggggaccagacagccgcgattggattaggtacaatcagttccgcagggagctgacattgactgtgctcgacatcgtgtccctcttcccgaactacgattcccgcacctacccaatccgcaccgtgtcccagctgacaagggagatctacactaatcccgtgctcgagaacttcgacggatccttcaggggctcggcacagggaattgagggatcaatccgctccccgcacctcatggacatcctcaacagcataacaatctacactgacgctcacaggggcgagtactattggtcggggcatcagatcatggcatcgcctgtgggcttctccggaccagagttcacctttcctctgtacggcacgatgggaaacgcggcgccgcagcaaaggatcgttgcccagctgggacaaggagtgtaccgcaccctctcctccaccctctatcgccgcccgttcaacattggcatcaacaaccagcaactgtctgtgctcgacggcaccgagttcgcctacggcacctcctccaacctcccgtcagcggtctataggaagtcaggcaccgttgactccctcgacgagatcccgccccagaacaataacgtgccacctaggcaaggcttctcgcaccggctctcccatgtcagcatgttccgctcgggcttctccaactcatccgtgtccatcatcagggccccgatgttctcctggatccacaggtccgccgagttcaacaacattataccatccagccagatcacacaaattcctctgaccaagtccacgaacctcggttcaggcacctccgtggtgaagggaccagggttcaccggcggggatatcctgcgcaggacgtcgcctggccagatatccaccctccgcgtcaatatcaccgccccgctcagccaacgctaccgcgtgcgcatccgctatgcgtcaacaactaacctccagttccacacatccatcgacggccggcccattaatcaagggaacttctcggctaccatgtcgtctggctccaacctccagtcggggtctttccgcacggtcggcttcaccacgccattcaatttctccaacggctcctccgtgttcacgctctctgcgcatgtgttcaactcaggcaacgaggtttacatagatcgcatcgagttcgtcccggccgaggttacattcgaggcagaatacgacctggagagggctcagaaagcagtgaacgagctgttcaccagctctaaccagattgggctgaagaccgacgtgaccgactaccacattgaccaggtgtccaacttggtggagtgcctgagcgacgagttctgcctcgacgagaagaaggaactgtcggagaaggtgaagcacgccaagcggctcagcgatgagcgcaaccttctccaggacccgaatttcagggggatcaaccgccagctggacaggggctggcgcggctccaccgacatcacgatccagggcggcgatgacgtgttcaaggagaactacgtgaccctgctcggcactttcgacgagtgctaccccacctacctgtaccagaagatcgacgagtccaagctgaaggcctacactcgctaccaactccgcggttacatcgaagactcccaggacctggagatttacctgatccgctacaatgccaagcacgagacggtcaacgtgccgggcaccggctcgctgtggcccctcagcgctcccagcccgatcggcaagtgcgcccaccacagccaccacttctccctcgacatcgacgtgggctgcaccgacctcaacgaggacctgggagtctgggtcatcttcaagatcaagacgcaggacggacacgcacgcctgggcaaccttgagttcctggaagagaagccgctggtcggggaggctctggcgcgtgtcaagcgcgcagagaagaagtggagggacaaacgcgagaagctcgaatgggagacgaacatcgtgtacaaggaggccaaggagtcggtggatgccttgtttgtgaactcccagtatgaccgcctgcaagcggacaccaacatcgccatgatccacgctgccgacaagagggtgcactccatcagggaggcctacctccctgagctgtccgtgatcccaggcgtcaacgccgcgatcttcgaggaactggagggccgcatcttcaccgcattctcgctctacgacgctcgcaacgtcatcaagaacggcgacttcaataacgggctgtcctgctggaacgtgaagggccatgtggacgtggaagagcagaataaccacaggtcggtcctggtcgtgccggagtgggaagccgaggtgtcccaggaggttcgcgtctgccccggtcggggctacattctgcgcgtgacggcctacaaggagggctacggtgaggggtgcgtcaccatccacgagatcgagaacaacaccgatgaactcaagttcagcaactgcgtcgaagaggaggtctacccgaacaataccgttacgtgcaacgactacaccgccacacaggaggaatacgagggcacttacacctcccgcaaccgtggctacgacggcgcgtacgagtccaactcgtccgttcccgccgactatgcctccgcttacgaagagaaagcctacaccgatggcaggcgcgacaacccttgcgagagcaaccgcggctacggggactacaccccgttgccagccggctacgttaccaaggaactcgaatactttcccgagacggacaaggtgtggatcgagatcggcgagacggaggggaccttcatcgtggactccgtcgagcttctgctcatggaagagtaatgactagctatatcatcaatttatgtattacacataatatcgcactcagtctttcatctacggcaatgtaccagctgatataatcagttattgaaatatttctgaatttaaacttgcatcaataaatttatgtttttgcttggactataatacctgacttgttattttatcaataaatatttaaactatatttctttcaagatatcattctttacaagtatacgtgtttaaattgaataccataaatttttatttttcaaatacatgtaaaattatgaaatgggagtggtggcgaccgagctcaagcacacttcaattcctataacggaccaaatcgcaaaaattataataacatattatttcatcctggattaaaagaaagtcaccggggattattttgtgacgccgattacatacggcgacaataaagacattggaaatcgtagtacatattggaatacactgattatattaatgatgaatacatactttaatatccttacgtaggatcccgatcctacctgtcacttcatcaaaaggacagtagaaaaggaaggtggcacctacaaatgccatcattgcgataaaggaaaggctatcattcaagatgcctctgccgacagtggtcccaaagatggacccccacccacgaggagcatcgtggaaaaagaagacgttccaaccacgtcttcaaagcaagtggattgatgtgatacttccactgacgtaagggatgacgcacaatcccactatccttcgcaagacccttcctctatataaggaagttcatttcatttggagaggaccatgtcgcccgagcgcaggcccgtcgagatccgcccggccacagcagccgacatggctgcggtgtgcgacatcgtcaaccactacatcgaaacgtccaccgtgaacttccgcaccgagccgcagacgccgcaggagtggatcgacgaccttgagcgcctccaggaccgctacccctggctcgtcgcggaggtcgaaggcgtcgtggccggcatcgcctacgccgggccgtggaaggctcgcaacgcctacgactggaccgtcgagagcaccgtctacgtgtcccaccgccaccagcgcctgggcctcggctccacgctgtacacgcacctgctcaagtcgatggaggcgcaaggcttcaagagcgtggtcgccgtcatcggcctcccgaacgatccctccgtgaggctccacgaagccctgggctacaccgctcggggcacgctgcgcgcagccggctacaagcacggtggctggcacgacgtcgggttctggcagagggacttcgagctgcccgcgcctccgcgcccggttcgccccgtgacccagatttgatagtttctccataataatgtgtgagtagttcccagataagggaattagggttcctatagggtttcgctcatgtgttgagcatataagaaacccttagtatgtatttgtatttgtaaaatacttctatcaataaaatttctaattcctaaaaccaaaatccagtactaaaatccagatcgggcccactagtgaattcccccgaattaattcggcgttaattcagtacattaaaaacg

SEQ ID NO: 10 - DNA, 14760 bp, Zea mays
  source 1..14760: mol_type = genomic DNA
cgaagctacggtcgaggggttagcgcgtttacgttaaacaagtactaattagaacatctaattcaacataattatattaattgatattaatcaaatgtaaattaatactactacttagttttgactaacttactattttaatagttgacaattaagcaagtaacttaatgaatatgagtgattctaagcgagacgaattaacgacgcacgacatgcaaacacgatgtgcgcaacgcgcggacacaaacgacttagcacgcggacaacgcgcgatacgcgcgaacggcacgcggcaatgcgcgcgacacacgcgaacgacacgcgacaacgcgcggacacttgcaaacgacatgcgtgaaacagcaccgcggcacgcgcacggtacgcgcggaccgacatgcgaaactaataaataaatgacaacgtgattacactaaacaattattaatatgtaacatttcagttaaggttaatcatattggtgactaattataaatgcgcgaatcgaattcctaaattagatttttaaattgaaatgtcgttttagtagccactggttaaacaaacgtttaactaaattaaataaaatgtgcaaaaattgggataaatatttctaaattaagattattttaatacgaatctaacgcaacttgaatggatcaaatcggatttaaaacgcaaaacttatgaatgttttaaaccatactgtaattcgcgcgtagtttaaactgaaggcgggaaacgacaatctgatccaagctcaagctgctaagcttattcgggtcaaggcggaagccagcgcgccaccccacgtcagcaaatacggaggcgcggggttgacggcgtcacccggtcctaacggcgaccaacaaaccagccagaagaaattacagtaaaaaaaaagtaaattgcactttgatccaccttttattacctaagtctcaatttggatcacccttaaacctatcttttcaatttgggccgggttgtggtttggactaccatgaacaacttttcgtcatgtctaacttccctttcagcaaacatatgaacaatatatagagaagatcggccgtatactagagctgatgtgtttaaggtcgttgattgcacgagaaaaaaaaatccaaatcgcaacaatagcaaatttatctggttcaaagtgaaaagatatgtttaaaggtagtccaaagtaaaacttatagataataaaatgtggtccaaagcgtaattcactcaaaaaaaatcaacgagacgtgtaccaaacggagacaaacggcatcttctcgaaatttcccaaccgctcgctcgcccgcctcgtcttcccggaaaccgcggtggtttcagcgtggcggattctccaagcagacggagacgtcacggcacgggactcctcccaccacccaaccgccataaataccagccccctcatctcctctcctcgcatcagctccacccccgaaaaatttctccccaatctcgcgaggctctcgtcgtcgaatcgaatcctctcgcgtcctcaaggtacgctgcttctcctctcctcgcttcgtttcgattcgatttcggacgggtgaggttgttttgttgctagatccgattggtggttagggttgtcgatgtgattatcgtgagatgtttaggggttgtagatctgatggttgtgatttgggcacggttggttcgataggtggaatcgtggttaggttttgggattgggatgttggttctgatgattggggggaatttttacggttagatgaattgttggatgattcgattggggaaatcggtgtagatctgttggggaattgtggaactagtcatgcctgagtgattggtgcgatttgtagcgtgttccatcttgtaggccttgttgcgagcatgttcagatctactgttccgctcttgattgagttattggtgccatgggttggtgcaaacacaggctttaatatgttatatctgttttgtgtttgatgtagatctgtagggtagttcttcttagacatggttcaattatgtagcttgtgcgtttcgatttgatttcatatgttcacagattagataatgatgaactcttttaattaattgtcaatggtaaataggaagtcttgtcgctatatctgtcataatgatctcatgttactatctgccagtaatttatgctaagaactatattagaatatcatgttacaatctgtagtaatatcatgttacaatctgtagttcatctatataatctattgtggtaatttctttttactatctgtgtgaagattattgccactagttcattctacttatttctgaagttcaggatacgtgtgctgttactacctatctgaatacatccgtgatgtgcctgttactatctttttgaatacatgtatgttctgttggaatatgtttgctgtttgatccgttgttgtgtccttaatcttgtgctagttcttaccctatctgtttggtgattatttcttgcagaccatggcgcccaccgtgatgatggcctcgtcggccaccgccgtcgcttcgttccaggggctcaagtccaccgccagcctccccgtcgcccgccgctcctccagaagcctcggcaacgtcagcaacggcggaaggatccggtgcatgcaggtgtggccggcctacggcaacaagaagttcgagacgctgtcgtacctgccgccgctgtccaccggcgggcgcatccgctgcatgcaggccatgaacaagaacaacacgaagctctccacccgcggcctgcaaagcttcatcgactacttcaacggcatctacggcttcgcgaccggcatcaaggacatcatgaacatgatcttcaagacggacacgggcggcgacctgacgctcgacgagatcctcaagaaccagcagctcctgaacgacatctcgggcaagctggacggcgtgaacggctccctgaacgacctcatcgcccagggcaacctcaacaccgagctgagcaaggagatcctcaagatcgcgaacgagcagaaccaggtgctgaacgacgtcaacaacaagctcgacgccatcaacaccatgctccgcgtgtacctgcccaagatcacgtccatgctcagcgacgtcatcaagcagaactacgccctgtccctccagatcgagtacctcagcaagcagctgcaggagatctccgacaagctggacatcatcaacgtgaacgtcctcatcaactccaccctgacggagatcaccccggcgtaccagcgcatcaagtatgtgaacgagaagttcgaggagctgacgttcgccaccgagacgtccagcaaggtcaagaaggacggcagccccgccgacatcctggacgagctgaccgagctgacggagctggcgaagtccgtgaccaagaacgacgtcgacggcttcgagttctacctgaacacgttccacgacgtgatggtcggcaacaacctcttcggcaggtcggctctgaagaccgccagcgagctgatcaccaaggagaacgtgaagacgtccggcagcgaagtgggcaacgtctacaacttcctgatcgtcctcacggccctgcaggctcaggcgttcctgaccctgacgacctgccgcaagctcctgggcctcgctgacatcgactacaccagcatcatgaacgagcacctgaacaaggagaaggaggagttcagggtgaacatcctcccgaccctgtccaacacgttcagcaaccccaactacgccaaggtgaagggctccgacgaggacgcgaagatgatcgtggaggctaagcccggccacgccctcatcggcttcgagatctccaacgacagcatcaccgtgctgaaggtctacgaggcgaagctcaagcagaactaccaggtggacaaggactccctgagcgaggtcatctacggcgacatggacaagctcctgtgcccggaccagagcgagcagatctactacaccaacaacatcgtgttccccaacgagtatgtgatcaccaagatcgacttcacgaagaagatgaagaccctccgctacgaggtgaccgccaacttctacgactccagcacgggcgagatcgacctcaacaagaagaaggtcgagtccagcgaggccgagtacaggaccctgagcgcgaacgacgacggcgtgtacatgccgctgggcgtcatctccgagacgttcctcacccccatcaacggcttcggcctgcaggccgacgagaacagccgcctcatcaccctgacgtgcaagtcctacctcagggagctgctgctcgccaccgacctgagcaacaaggagacgaagctcatcgtgccgccctccggcttcatcagcaacatcgtcgagaacggctccatcgaggaggacaacctggagccctggaaggccaacaacaagaacgcctacgtggaccacaccggcggcgtcaacggcacgaaggcgctctacgtgcacaaggacggtggcatcagccagttcatcggcgacaagctgaagccgaagaccgagtatgtgatccagtacacggtcaagggcaagccctccatccacctgaaggacgagaacaccggctacatccactacgaggacacgaacaacaacctcgaggactaccagaccatcaacaagcgcttcaccacgggcacggacctgaagggcgtctacctgatcctcaagtcccagaacggcgacgaggcgtggggcgacaacttcatcatcctcgagatctcgccctcggagaagctgctcagcccggagctgatcaacaccaacaactggacctccacgggcagcacgaacatctccggcaacacgctgaccctctaccagggcggcaggggcatcctcaagcagaacctgcagctcgactccttcagcacctacagggtgtacttctccgtcagcggcgacgcgaacgtgcgcatcaggaactcccgcgaggtcctgttcgagaagaggtacatgtccggcgccaaggacgtgagcgagatgttcaccacgaagttcgagaaggacaacttctacatcgagctgagccagggcaacaacctctacggtggcccgatcgtgcacttctacgacgtctccatcaagtagtgactaggctactgtagctagctgtgcatgtatgtggtgtggttactaaaataattagtgttttccttttgtttggaagcatatgtgtggtgaataaatgatgaactccgatgttcctctctataaatcttgatgattcgctagctatccgtacgtcgttgttctttgatttgatgatgagattgaaaaatggaatgtcatgctaaggagggtgccggtaccgcattccagattgggttcaatcaacaaggtacgagccatatcactttattcaaattggtatcgccaaaaccaagaaggaactcccatcctcaaaggtttgtaaggaagaattctcagtccaaagcctcaacaaggtcagggtacagagtctccaaaccattagccaaaagctacaggagatcaatgaagaatcttcaatcaaagtaaactactgttccagcacatgcatcatggtcagtaagtttcagaaaaagacatccaccgaagacttaaagttagtgggcatctttgaaagtaatcttgtcaacatcgagcagctggcttgtggggaccagacaaaaaaggaatggtgcagaattgttaggcgcacctaccaaaagcatctttgcctttattgcaaagataaagcagattcctctagtacaagtggggaacaaaataacgtggaaaagagctgtcctgacagcccactcactaatgcgtatgacgaacgcagtgacgaccacaaaagaattccctctatataagaaggcattcattcccatttgaaggatcatcagatactcaaccaatccttctaggatctaccgtcttcggtacgcgctcactccgccctctgcctttgttactgccacgtttctctgaatgctctcttgtgtggtgattgctgagagtggtttagctggatctagaattacactctgaaatcgtgttctgcctgtgctgattacttgccgtcctttgtagcagcaaaatatagggacatggtagtacgaaacgaagatagaacctacacagcaatacgagaaatgtgtaatttggtgcttagcggtatttatttaagcacatgttggtgttatagggcacttggattcagaagtttgctgttaatttaggcacaggcttcatactacatgggtcaatagtatagggattcatattataggcgatactataataatttgttcgtctgcagagcttattatttgccaaaattagatattcctattctgtttttgtttgtgtgctgttaaattgttaacgcctgaaggaataaatataaatgacgaaattttgatgtttatctctgctcctttattgtgaccataagtcaagatcagatgcacttgttttaaatattgttgtctgaagaaataagtactgacagtattttgatgcattgatctgcttgtttgttgtaacaaaatttaaaaataaagagtttcctttttgttgctctccttacctcctgatggtatctagtatctaccaactgacactatattgcttctctttacatacgtatcttgctcgatgccttctccctagtgttgaccagtgttactcacatagtctttgctcatttcattgtaatgcagataccaagcggaccatggcgcaagttagcaggatctgcaacggcgtgcagaacccgtcgctcatctccaacctctcgaaatccagtcaacgcaaatcgcccttgtcggtgtccctgaagacgcagcagcacccgcgagcctacccgatctcgtcgtcgtggggcttgaagaagagcgggatgacgctgattggctctgagctccgtcccctcaaggtcatgtcttctgtgtccacggcgtgcatggataataaccctaacatcaatgagtgcattccctacaactgcctgtctaacccagaggtggaggtgctcggcggggagaggattgagacgggctacacgcccatcgacatttccctcagcctgacccagttcctcctgtccgaatttgtcccaggtgccggattcgtgctcggcctcgtcgatatcatttggggtatcttcggaccgagccagtgggacgccttcctcgtgcagattgagcaactcatcaaccagcgcatcgaggaattcgccaggaaccaagcgatttcccgcctcgagggcctctccaacctctaccagatctacgccgaatccttcagggagtgggaagcggatcccaccaacccggccctgagggaggaaatgagaattcagttcaatgacatgaacagcgctttgaccacggcaatcccgctctttgcggtgcagaattaccaggtgccgcttttgtcggtctacgtgcaggccgcgaacctccacctgagcgtcctgagagatgtctcggttttcggtcagcgctggggatttgacgctgcaaccattaattcccgctacaacgacctcacacgcctcatcggcaattacactgaccatgccgtgaggtggtataacaccggcctcgagagggtctggggaccagacagccgcgattggattaggtacaatcagttccgcagggagctgacattgactgtgctcgacatcgtgtccctcttcccgaactacgattcccgcacctacccaatccgcaccgtgtcccagctgacaagggagatctacactaatcccgtgctcgagaacttcgacggatccttcaggggctcggcacagggaattgagggatcaatccgctccccgcacctcatggacatcctcaacagcataacaatctacactgacgctcacaggggcgagtactattggtcggggcatcagatcatggcatcgcctgtgggcttctccggaccagagttcacctttcctctgtacggcacgatgggaaacgcggcgccgcagcaaaggatcgttgcccagctgggacaaggagtgtaccgcaccctctcctccaccctctatcgccgcccgttcaacattggcatcaacaaccagcaactgtctgtgctcgacggcaccgagttcgcctacggcacctcctccaacctcccgtcagcggtctataggaagtcaggcaccgttgactccctcgacgagatcccgccccagaacaataacgtgccacctaggcaaggcttctcgcaccggctctcccatgtcagcatgttccgctcgggcttctccaactcatccgtgtccatcatcagggccccgatgttctcctggatccacaggtccgccgagttcaacaacattataccatccagccagatcacacaaattcctctgaccaagtccacgaacctcggttcaggcacctccgtggtgaagggaccagggttcaccggcggggatatcctgcgcaggacgtcgcctggccagatatccaccctccgcgtcaatatcaccgccccgctcagccaacgctaccgcgtgcgcatccgctatgcgtcaacaactaacctccagttccacacatccatcgacggccggcccattaatcaagggaacttctcggctaccatgtcgtctggctccaacctccagtcggggtctttccgcacggtcggcttcaccacgccattcaatttctccaacggctcctccgtgttcacgctctctgcgcatgtgttcaactcaggcaacgaggtttacatagatcgcatcgagttcgtcccggccgaggttacattcgaggcagaatacgacctggagagggctcagaaagcagtgaacgagctgttcaccagctctaaccagattgggctgaagaccgacgtgaccgactaccacattgaccaggtgtccaacttggtggagtgcctgagcgacgagttctgcctcgacgagaagaaggaactgtcggagaaggtgaagcacgccaagcggctcagcgatgagcgcaaccttctccaggacccgaatttcagggggatcaaccgccagctggacaggggctggcgcggctccaccgacatcacgatccagggcggcgatgacgtgttcaaggagaactacgtgaccctgctcggcactttcgacgagtgctaccccacctacctgtaccagaagatcgacgagtccaagctgaaggcctacactcgctaccaactccgcggttacatcgaagactcccaggacctggagatttacctgatccgctacaatgccaagcacgagacggtcaacgtgccgggcaccggctcgctgtggcccctcagcgctcccagcccgatcggcaagtgcgcccaccacagccaccacttctccctcgacatcgacgtgggctgcaccgacctcaacgaggacctgggagtctgggtcatcttcaagatcaagacgcaggacggacacgcacgcctgggcaaccttgagttcctggaagagaagccgctggtcggggaggctctggcgcgtgtcaagcgcgcagagaagaagtggagggacaaacgcgagaagctcgaatgggagacgaacatcgtgtacaaggaggccaaggagtcggtggatgccttgtttgtgaactcccagtatgaccgcctgcaagcggacaccaacatcgccatgatccacgctgccgacaagagggtgcactccatcagggaggcctacctccctgagctgtccgtgatcccaggcgtcaacgccgcgatcttcgaggaactggagggccgcatcttcaccgcattctcgctctacgacgctcgcaacgtcatcaagaacggcgacttcaataacgggctgtcctgctggaacgtgaagggccatgtggacgtggaagagcagaataaccacaggtcggtcctggtcgtgccggagtgggaagccgaggtgtcccaggaggttcgcgtctgccccggtcggggctacattctgcgcgtgacggcctacaaggagggctacggtgaggggtgcgtcaccatccacgagatcgagaacaacaccgatgaactcaagttcagcaactgcgtcgaagaggaggtctacccgaacaataccgttacgtgcaacgactacaccgccacacaggaggaatacgagggcacttacacctcccgcaaccgtggctacgacggcgcgtacgagtccaactcgtccgttcccgccgactatgcctccgcttacgaagagaaagcctacaccgatggcaggcgcgacaacccttgcgagagcaaccgcggctacggggactacaccccgttgccagccggctacgttaccaaggaactcgaatactttcccgagacggacaaggtgtggatcgagatcggcgagacggaggggaccttcatcgtggactccgtcgagcttctgctcatggaagagtaatgactagctatatcatcaatttatgtattacacataatatcgcactcagtctttcatctacggcaatgtaccagctgatataatcagttattgaaatatttctgaatttaaacttgcatcaataaatttatgtttttgcttggactataatacctgacttgttattttatcaataaatatttaaactatatttctttcaagatatcattctttacaagtatacgtgtttaaattgaataccataaatttttatttttcaaatacatgtaaaattatgaaatgggagtggtggcgaccgagctcaagcacacttcaattcctataacggaccaaatcgcaaaaattataataacatattatttcatcctggattaaaagaaagtcaccggggattattttgtgacgccgattacatacggcgacaataaagacattggaaatcgtagtacatattggaatacactgattatattaatgatgaatacatactttaatatccttacgtaggatcccgatcctacctgtcacttcatcaaaaggacagtagaaaaggaaggtggcacctacaaatgccatcattgcgataaaggaaaggctatcattcaagatgcctctgccgacagtggtcccaaagatggacccccacccacgaggagcatcgtggaaaaagaagacgttccaaccacgtcttcaaagcaagtggattgatgtgatacttccactgacgtaagggatgacgcacaatcccactatccttcgcaagacccttcctctatataaggaagttcatttcatttggagaggaccatgtcgcccgagcgcaggcccgtcgagatccgcccggccacagcagccgacatggctgcggtgtgcgacatcgtcaaccactacatcgaaacgtccaccgtgaacttccgcaccgagccgcagacgccgcaggagtggatcgacgaccttgagcgcctccaggaccgctacccctggctcgtcgcggaggtcgaaggcgtcgtggccggcatcgcctacgccgggccgtggaaggctcgcaacgcctacgactggaccgtcgagagcaccgtctacgtgtcccaccgccaccagcgcctgggcctcggctccacgctgtacacgcacctgctcaagtcgatggaggcgcaaggcttcaagagcgtggtcgccgtcatcggcctcccgaacgatccctccgtgaggctccacgaagccctgggctacaccgctcggggcacgctgcgcgcagccggctacaagcacggtggctggcacgacgtcgggttctggcagagggacttcgagctgcccgcgcctccgcgcccggttcgccccgtgacccagatttgatagtttctccataataatgtgtgagtagttcccagataagggaattagggttcctatagggtttcgctcatgtgttgagcatataagaaacccttagtatgtatttgtatttgtaaaatacttctatcaataaaatttctaattcctaaaaccaaaatccagtactaaaatccagatcgggcccactagtgaattcccccgaattaattcggcgttaattcagtacattaaaaacgaccacacgcgaacgacacgcgacaacgcgcggacacttgcaaacgacatgcgtgaaacagcaccgcggcacgcgcacggtacgcgcggaccgacatgcgaaactaataaataaatgacaacgtgattacactaaacaattattaatatgtaacatttcagttaaggttaatcatattggtgactaattataaatgcgcgaatcgaattcctaaattagatttttaaattgaaatgtcgttttagtagccactggttaaacaaacgtttaactaaattaaataaaatgtgcaaaaattgggataaatatttctaaattaagattattttaatacgaatctaacgcaacttgaatggatcaaatcggatttaaaacgcaaaacttatgaatgttttaaaccatactgtaattcgcgcgtcctaatttacagaactgccatcttcttcttcctctcctcatcttcttcctcccatccatggaagagagaggaggggaagggggctgcgcaggggaggacgagaccgggccggccgggggcgggcgcggccgcaccgggcgcgcggggcgcggccacagccgccggggaggggtgcgcgcgggcgtggggcgcgtgagcgcgagcgccaccgccggccaccgccgccgccgccggggagggagaaaggggcgccgtcgaggaggggaaacagaggggggaggggcgccgccaccggggaaggtgaggggagagtgggagaggctctgcacggacgggaaaacgaaaaaaacgaagaaaccctaggtgcaacaatggaggtttctcaccggggaagaagaccctcgccggagccgaggagaaatccgtcgattgccggagattcggggatccaatcgatgaaccgaacgcgctgcgacgaagccttcgacgagacgaacgcagcggtactctcggattctgcagacgatgcacggattgggagtaattgctcgccggagttgtcgccggagttggaaccgccccgaacttcggcgagcaataccgggagctagggattggatttgggggaaacgtttggtgttctggaacgggctcgacgagataaagccggacatgtatatatacctagggtttggacgagacaaaaattcggattttattatttttaaaattcgaaaaagcctagaaatccatattttgtgctcaaaatattatagatactttcaaaaattccagaaaaattcctataaatgttttggcacctaatgaactcaaaaaacataattagaatttctaaaaacatttttaggttccacaaataaatggattttggtttccggaaaatagaaaaatattccgaaaaatatgaaaatttaccgagcgcttctataagatatgttaacatatttgaaacacattttacacttagaaacaccatgcaacgacatgaatgcaacaaccaaagtgcctctagggctcattccactaggtttacgctaatataaaacaaaatgattctccatttttaggaaaaagagaaaggaaagcgaagaactgagagagtaacacctgaatttggtggatattagaaaagaaattttatacccccaaattcagggtgttacaggtgaggagcttaggataatgttatttaactatagggagatgggaattattcctaaggttgagccgatgtaaagtgtggtgccctcgcttgtacatgtgtaaaggcttgtatgttgtgtgcccccgcacacttggctatgcttgcgaaggcgttatgtacttggtctggtgtattttgttatattgtgctggtgcgcatatagtcggtcttggcgcggacagtttggtgtggtcgtttttgcttttgttgtgctagtccggctgcacccttaggcgacttctgcacggatggtcgtcgcggtagacttcggtttttcgcacttgttgtgctagtccggctgcacccttaggcgacttctgcacagatagtcttcgcggtagacttcggtttttcgcacttgttgtgctagtccggctgcacccttaggcgacttctgcacggatagtcttcgcggtagacttcggtttttcgcacttgttgtgctagtccgactgcacccttaggcgacttctgcacggatagtcttcgcggtagacttcggtttttcgcacttgttgtgctagtccgactgcacccttaggcgacttctgcacagatagtcttcgcggtagacttcagtttttcgcacttgttgtgctagtccggctgcacccttaggcgacttctgcacggatagtcttcgcggtagacttaggtttttcgcacttgttgtgctattccggctgcacccttaggcgacttctgcgtggatttgtcgcacgcgagggtggctagcgctgagcctcgcggtgacctcgtattggtcgaatgtcgaagaccgtcgtcgcggtcttttttcgacgcatgtttttgcgggggatttttcatacatatattacatggctccgcctcgttaaaaacctcaccccccgggaggaaaagagtgcgggccagaataagattgtttttgcgaattacaagggcgaatcagccctgatgagtcaaacaaaaaatttgcggaggttgtcgatgttccaggagtgctccaggtcttcgccgtttggcgttgtgagcctgtaagcgctgcgggaagctttcgtcttgactatgaaggggccctcccacctgggctccagcttgcccctggactctgttcgagctgttcggatgagtac

SEQ ID NO: 11 - DNA, 1068 bp, Zea mays
  source 1..1068: mol_type = genomic DNA
cgacgcacgacatgcaaacacgatgtgcgcaacgcgcggacacaaacgacttagcacgcggacaacgcgcgatacgcgcgaacggcacgcggcaatgcgcgcgacacacgcgaacgacacgcgacaacgcgcggacacttgcaaacgacatgcgtgaaacagcaccgcggcacgcgcacggtacgcgcggaccgacatgcgaaactaataaataaatgacaacgtgattacactaaacaattattaatatgtaacatttcagttaaggttaatcatattggtgactaattataaatgcgcgaatcgaattcctaaattagatttttaaattgaaatgtcgttttagtagccactggttaaacaaacgtttaactaaattaaataaaatgtgcaaaaattgggataaatatttctaaattaagattattttaatacgaatctaacgcaacttgaatggatcaaatcggatttaaaacgcaaaacttatgaatgttttaaaccatactgtaattcgcgcgtagtttaaactgaaggcgggaaacgacaatctgatccaagctcaagctgctaagcttattcgggtcaaggcggaagccagcgcgccaccccacgtcagcaaatacggaggcgcggggttgacggcgtcacccggtcctaacggcgaccaacaaaccagccagaagaaattacagtaaaaaaaaagtaaattgcactttgatccaccttttattacctaagtctcaatttggatcacccttaaacctatcttttcaatttgggccgggttgtggtttggactaccatgaacaacttttcgtcatgtctaacttccctttcagcaaacatatgaacaatatatagagaagatcggccgtatactagagctgatgtgtttaaggtcgttgattgcacgagaaaaaaaaatccaaatcgcaacaatagcaaatttatctggttcaaagtgaaaagatatgtttaaaggtagtccaaagtaaaacttatagataataaaatgtggtccaaagcgtaattcactcaaaaaaaatcaacgagacgtgtaccaaacgg

SEQ ID NO: 12 - DNA, 798 bp, Zea mays
  source 1..798: mol_type = genomic DNA
ctggcagagggacttcgagctgcccgcgcctccgcgcccggttcgccccgtgacccagatttgatagtttctccataataatgtgtgagtagttcccagataagggaattagggttcctatagggtttcgctcatgtgttgagcatataagaaacccttagtatgtatttgtatttgtaaaatacttctatcaataaaatttctaattcctaaaaccaaaatccagtactaaaatccagatcgggcccactagtgaattcccccgaattaattcggcgttaattcagtacattaaaaacgaccacacgcgaacgacacgcgacaacgcgcggacacttgcaaacgacatgcgtgaaacagcaccgcggcacgcgcacggtacgcgcggaccgacatgcgaaactaataaataaatgacaacgtgattacactaaacaattattaatatgtaacatttcagttaaggttaatcatattggtgactaattataaatgcgcgaatcgaattcctaaattagatttttaaattgaaatgtcgttttagtagccactggttaaacaaacgtttaactaaattaaataaaatgtgcaaaaattgggataaatatttctaaattaagattattttaatacgaatctaacgcaacttgaatggatcaaatcggatttaaaacgcaaaacttatgaatgttttaaaccatactgtaattcgcgcgtcctaatttacagaactgccatcttcttcttcctctcctcatcttcttcctcccatccatggaagagagaggaggggaaggg

SEQ ID NO: 13 - DNA, 20 bp, synthetic construct
  source 1..20: mol_type = other DNA
cgacgcacgacatgcaaaca

SEQ ID NO: 14 - DNA, 20 bp, synthetic construct
  source 1..20: mol_type = other DNA
ccgtttggtacacgtctcgt

SEQ ID NO: 15 - DNA, 20 bp, synthetic construct
  source 1..20: mol_type = other DNA
cccttcccctcctctctctt

SEQ ID NO: 16 - DNA, 21 bp, synthetic construct
  source 1..21: mol_type = other DNA
ctggcagagggacttcgagct

SEQ ID NO: 17 - DNA, 22 bp, synthetic construct
  source 1..22: mol_type = other DNA
gctgtttgatccgttgttgtgt

SEQ ID NO: 18 - DNA, 20 bp, synthetic construct
  source 1..20: mol_type = other DNA
gaggatctccttgctcagct

SEQ ID NO: 19 - DNA, 20 bp, synthetic construct
  source 1..20: mol_type = other DNA
gccttctccctagtgttgac

SEQ ID NO: 20 - DNA, 20 bp, synthetic construct
  source 1..20: mol_type = other DNA
cgctggttgatgagttgctc

SEQ ID NO: 21 - DNA, 20 bp, synthetic construct
  source 1..20: mol_type = other DNA
cccgatcctacctgtcactt

SEQ ID NO: 22 - DNA, 20 bp, synthetic construct
  source 1..20: mol_type = other DNA
ctctgccagaacccgacgtc

SEQ ID NO: 23 - DNA, 23 bp, synthetic construct
  source 1..23: mol_type = other DNA
gaacaagaacaacacgaagctct

SEQ ID NO: 24 - DNA, 23 bp, synthetic construct
  source 1..23: mol_type = other DNA
cttgatggagacgtcgtagaagt

SEQ ID NO: 25 - DNA, 22 bp, synthetic construct
  source 1..22: mol_type = other DNA
cattccctacaactgcctgtct

SEQ ID NO: 26 - DNA, 25 bp, synthetic construct
  source 1..25: mol_type = other DNA
cattactcttccatgagcagaagct

SEQ ID NO: 27 - DNA, 20 bp, synthetic construct
  source 1..20: mol_type = other DNA
gtgcgacatcgtcaaccact

SEQ ID NO: 28 - DNA, 20 bp, synthetic construct
  source 1..20: mol_type = other DNA
ctctgccagaacccgacgtc

SEQ ID NO: 29 - DNA, 1708 bp, synthetic construct
  source 1..1708: mol_type = other DNA
attcgggtcaaggcggaagccagcgcgccaccccacgtcagcaaatacggaggcgcggggttgacggcgtcacccggtcctaacggcgaccaacaaaccagccagaagaaattacagtaaaaaaaaagtaaattgcactttgatccaccttttattacctaagtctcaatttggatcacccttaaacctatcttttcaatttgggccgggttgtggtttggactaccatgaacaacttttcgtcatgtctaacttccctttcagcaaacatatgaacaatatatagagaagatcggccgtatactagagctgatgtgtttaaggtcgttgattgcacgagaaaaaaaaatccaaatcgcaacaatagcaaatttatctggttcaaagtgaaaagatatgtttaaaggtagtccaaagtaaaacttatagataataaaatgtggtccaaagcgtaattcactcaaaaaaaatcaacgagacgtgtaccaaacggagacaaacggcatcttctcgaaatttcccaaccgctcgctcgcccgcctcgtcttcccggaaaccgcggtggtttcagcgtggcggattctccaagcagacggagacgtcacggcacgggactcctcccaccacccaaccgccataaataccagccccctcatctcctctcctcgcatcagctccacccccgaaaaatttctccccaatctcgcgaggctctcgtcgtcgaatcgaatcctctcgcgtcctcaaggtacgctgcttctcctctcctcgcttcgtttcgattcgatttcggacgggtgaggttgttttgttgctagatccgattggtggttagggttgtcgatgtgattatcgtgagatgtttaggggttgtagatctgatggttgtgatttgggcacggttggttcgataggtggaatcgtggttaggttttgggattgggatgttggttctgatgattggggggaatttttacggttagatgaattgttggatgattcgattggggaaatcggtgtagatctgttggggaattgtggaactagtcatgcctgagtgattggtgcgatttgtagcgtgttccatcttgtaggccttgttgcgagcatgttcagatctactgttccgctcttgattgagttattggtgccatgggttggtgcaaacacaggctttaatatgttatatctgttttgtgtttgatgtagatctgtagggtagttcttcttagacatggttcaattatgtagcttgtgcgtttcgatttgatttcatatgttcacagattagataatgatgaactcttttaattaattgtcaatggtaaataggaagtcttgtcgctatatctgtcataatgatctcatgttactatctgccagtaatttatgctaagaactatattagaatatcatgttacaatctgtagtaatatcatgttacaatctgtagttcatctatataatctattgtggtaatttctttttactatctgtgtgaagattattgccactagttcattctacttatttctgaagttcaggatacgtgtgctgttactacctatctgaatacatccgtgatgtgcctgttactatctttttgaatacatgtatgttctgttggaatatgtttgctgtttgatccgttgttgtgtccttaatcttgtgctagttcttaccctatctgtttggtgattatttcttg

SEQ ID NO: 30 - DNA, 2373 bp, synthetic construct
  source 1..2373: mol_type = other DNA
atgaacaagaacaacacgaagctctccacccgcggcctgcaaagcttcatcgactacttcaacggcatctacggcttcgcgaccggcatcaaggacatcatgaacatgatcttcaagacggacacgggcggcgacctgacgctcgacgagatcctcaagaaccagcagctcctgaacgacatctcgggcaagctggacggcgtgaacggctccctgaacgacctcatcgcccagggcaacctcaacaccgagctgagcaaggagatcctcaagatcgcgaacgagcagaaccaggtgctgaacgacgtcaacaacaagctcgacgccatcaacaccatgctccgcgtgtacctgcccaagatcacgtccatgctcagcgacgtcatcaagcagaactacgccctgtccctccagatcgagtacctcagcaagcagctgcaggagatctccgacaagctggacatcatcaacgtgaacgtcctcatcaactccaccctgacggagatcaccccggcgtaccagcgcatcaagtatgtgaacgagaagttcgaggagctgacgttcgccaccgagacgtccagcaaggtcaagaaggacggcagccccgccgacatcctggacgagctgaccgagctgacggagctggcgaagtccgtgaccaagaacgacgtcgacggcttcgagttctacctgaacacgttccacgacgtgatggtcggcaacaacctcttcggcaggtcggctctgaagaccgccagcgagctgatcaccaaggagaacgtgaagacgtccggcagcgaagtgggcaacgtctacaacttcctgatcgtcctcacggccctgcaggctcaggcgttcctgaccctgacgacctgccgcaagctcctgggcctcgctgacatcgactacaccagcatcatgaacgagcacctgaacaaggagaaggaggagttcagggtgaacatcctcccgaccctgtccaacacgttcagcaaccccaactacgccaaggtgaagggctccgacgaggacgcgaagatgatcgtggaggctaagcccggccacgccctcatcggcttcgagatctccaacgacagcatcaccgtgctgaaggtctacgaggcgaagctcaagcagaactaccaggtggacaaggactccctgagcgaggtcatctacggcgacatggacaagctcctgtgcccggaccagagcgagcagatctactacaccaacaacatcgtgttccccaacgagtatgtgatcaccaagatcgacttcacgaagaagatgaagaccctccgctacgaggtgaccgccaacttctacgactccagcacgggcgagatcgacctcaacaagaagaaggtcgagtccagcgaggccgagtacaggaccctgagcgcgaacgacgacggcgtgtacatgccgctgggcgtcatctccgagacgttcctcacccccatcaacggcttcggcctgcaggccgacgagaacagccgcctcatcaccctgacgtgcaagtcctacctcagggagctgctgctcgccaccgacctgagcaacaaggagacgaagctcatcgtgccgccctccggcttcatcagcaacatcgtcgagaacggctccatcgaggaggacaacctggagccctggaaggccaacaacaagaacgcctacgtggaccacaccggcggcgtcaacggcacgaaggcgctctacgtgcacaaggacggtggcatcagccagttcatcggcgacaagctgaagccgaagaccgagtatgtgatccagtacacggtcaagggcaagccctccatccacctgaaggacgagaacaccggctacatccactacgaggacacgaacaacaacctcgaggactaccagaccatcaacaagcgcttcaccacgggcacggacctgaagggcgtctacctgatcctcaagtcccagaacggcgacgaggcgtggggcgacaacttcatcatcctcgagatctcgccctcggagaagctgctcagcccggagctgatcaacaccaacaactggacctccacgggcagcacgaacatctccggcaacacgctgaccctctaccagggcggcaggggcatcctcaagcagaacctgcagctcgactccttcagcacctacagggtgtacttctccgtcagcggcgacgcgaacgtgcgcatcaggaactcccgcgaggtcctgttcgagaagaggtacatgtccggcgccaaggacgtgagcgagatgttcaccacgaagttcgagaaggacaacttctacatcgagctgagccagggcaacaacctctacggtggcccgatcgtgcacttctacgacgtctccatcaagtagtga

SEQ ID NO: 31 - DNA, 237 bp, synthetic construct
  source 1..237: mol_type = other DNA
accatggcgcccaccgtgatgatggcctcgtcggccaccgccgtcgcttcgttccaggggctcaagtccaccgccagcctccccgtcgcccgccgctcctccagaagcctcggcaacgtcagcaacggcggaaggatccggtgcatgcaggtgtggccggcctacggcaacaagaagttcgagacgctgtcgtacctgccgccgctgtccaccggcgggcgcatccgctgcatgcag

SEQ ID NO: 32 - DNA, 213 bp, synthetic construct
  source 1..213: mol_type = other DNA
ctaggctactgtagctagctgtgcatgtatgtggtgtggttactaaaataattagtgttttccttttgtttggaagcatatgtgtggtgaataaatgatgaactccgatgttcctctctataaatcttgatgattcgctagctatccgtacgtcgttgttctttgatttgatgatgagattgaaaaatggaatgtcatgctaaggagggtgcc

SEQ ID NO: 33 - DNA, 565 bp, synthetic construct
  source 1..565: mol_type = other DNA
gcattccagattgggttcaatcaacaaggtacgagccatatcactttattcaaattggtatcgccaaaaccaagaaggaactcccatcctcaaaggtttgtaaggaagaattctcagtccaaagcctcaacaaggtcagggtacagagtctccaaaccattagccaaaagctacaggagatcaatgaagaatcttcaatcaaagtaaactactgttccagcacatgcatcatggtcagtaagtttcagaaaaagacatccaccgaagacttaaagttagtgggcatctttgaaagtaatcttgtcaacatcgagcagctggcttgtggggaccagacaaaaaaggaatggtgcagaattgttaggcgcacctaccaaaagcatctttgcctttattgcaaagataaagcagattcctctagtacaagtggggaacaaaataacgtggaaaagagctgtcctgacagcccactcactaatgcgtatgacgaacgcagtgacgaccacaaaagaattccctctatataagaaggcattcattcccatttgaaggatcatcagatact

SEQ ID NO: 34 - DNA, 3471 bp, synthetic construct
  source 1..3471: mol_type = other DNA
atggataataaccctaacatcaatgagtgcattccctacaactgcctgtctaacccagaggtggaggtgctcggcggggagaggattgagacgggctacacgcccatcgacatttccctcagcctgacccagttcctcctgtccgaatttgtcccaggtgccggattcgtgctcggcctcgtcgatatcatttggggtatcttcggaccgagccagtgggacgccttcctcgtgcagattgagcaactcatcaaccagcgcatcgaggaattcgccaggaaccaagcgatttcccgcctcgagggcctctccaacctctaccagatctacgccgaatccttcagggagtgggaagcggatcccaccaacccggccctgagggaggaaatgagaattcagttcaatgacatgaacagcgctttgaccacggcaatcccgctctttgcggtgcagaattaccaggtgccgcttttgtcggtctacgtgcaggccgcgaacctccacctgagcgtcctgagagatgtctcggttttcggtcagcgctggggatttgacgctgcaaccattaattcccgctacaacgacctcacacgcctcatcggcaattacactgaccatgccgtgaggtggtataacaccggcctcgagagggtctggggaccagacagccgcgattggattaggtacaatcagttccgcagggagctgacattgactgtgctcgacatcgtgtccctcttcccgaactacgattcccgcacctacccaatccgcaccgtgtcccagctgacaagggagatctacactaatcccgtgctcgagaacttcgacggatccttcaggggctcggcacagggaattgagggatcaatccgctccccgcacctcatggacatcctcaacagcataacaatctacactgacgctcacaggggcgagtactattggtcggggcatcagatcatggcatcgcctgtgggcttctccggaccagagttcacctttcctctgtacggcacgatgggaaacgcggcgccgcagcaaaggatcgttgcccagctgggacaaggagtgtaccgcaccctctcctccaccctctatcgccgcccgttcaacattggcatcaacaaccagcaactgtctgtgctcgacggcaccgagttcgcctacggcacctcctccaacctcccgtcagcggtctataggaagtcaggcaccgttgactccctcgacgagatcccgccccagaacaataacgtgccacctaggcaaggcttctcgcaccggctctcccatgtcagcatgttccgctcgggcttctccaactcatccgtgtccatcatcagggccccgatgttctcctggatccacaggtccgccgagttcaacaacattataccatccagccagatcacacaaattcctctgaccaagtccacgaacctcggttcaggcacctccgtggtgaagggaccagggttcaccggcggggatatcctgcgcaggacgtcgcctggccagatatccaccctccgcgtcaatatcaccgccccgctcagccaacgctaccgcgtgcgcatccgctatgcgtcaacaactaacctccagttccacacatccatcgacggccggcccattaatcaagggaacttctcggctaccatgtcgtctggctccaacctccagtcggggtctttccgcacggtcggcttcaccacgccattcaatttctccaacggctcctccgtgttcacgctctctgcgcatgtgttcaactcaggcaacgaggtttacatagatcgcatcgagttcgtcccggccgaggttacattcgaggcagaatacgacctggagagggctcagaaagcagtgaacgagctgttcaccagctctaaccagattgggctgaagaccgacgtgaccgactaccacattgaccaggtgtccaacttggtggagtgcctgagcgacgagttctgcctcgacgagaagaaggaactgtcggagaaggtgaagcacgccaagcggctcagcgatgagcgcaaccttctccaggacccgaatttcagggggatcaaccgccagctggacaggggctggcgcggctccaccgacatcacgatccagggcggcgatgacgtgttcaaggagaactacgtgaccctgctcggcactttcgacgagtgctaccccacctacctgtaccagaagatcgacgagtccaagctgaaggcctacactcgctaccaactccgcggttacatcgaagactcccaggacctggagatttacctgatccgctacaatgccaagcacgagacggtcaacgtgccgggcaccggctcgctgtggcccctcagcgctcccagcccgatcggcaagtgcgcccaccacagccaccacttctccctcgacatcgacgtgggctgcaccgacctcaacgaggacctgggagtctgggtcatcttcaagatcaagacgcaggacggacacgcacgcctgggcaaccttgagttcctggaagagaagccgctggtcggggaggctctggcgcgtgtcaagcgcgcagagaagaagtggagggacaaacgcgagaagctcgaatgggagacgaacatcgtgtacaaggaggccaaggagtcggtggatgccttgtttgtgaactcccagtatgaccgcctgcaagcggacaccaacatcgccatgatccacgctgccgacaagagggtgcactccatcagggaggcctacctccctgagctgtccgtgatcccaggcgtcaacgccgcgatcttcgaggaactggagggccgcatcttcaccgcattctcgctctacgacgctcgcaacgtcatcaagaacggcgacttcaataacgggctgtcctgctggaacgtgaagggccatgtggacgtggaagagcagaataaccacaggtcggtcctggtcgtgccggagtgggaagccgaggtgtcccaggaggttcgcgtctgccccggtcggggctacattctgcgcgtgacggcctacaaggagggctacggtgaggggtgcgtcaccatccacgagatcgagaacaacaccgatgaactcaagttcagcaactgcgtcgaagaggaggtctacccgaacaataccgttacgtgcaacgactacaccgccacacaggaggaatacgagggcacttacacctcccgcaaccgtggctacgacggcgcgtacgagtccaactcgtccgttcccgccgactatgcctccgcttacgaagagaaagcctacaccgatggcaggcgcgacaacccttgcgagagcaaccgcggctacggggactacaccccgttgccagccggctacgttaccaaggaactcgaatactttcccgagacggacaaggtgtggatcgagatcggcgagacggaggggaccttcatcgtggactccgtcgagcttctgctcatggaagagtaatga

SEQ ID NO: 35 - DNA, 804 bp, synthetic construct
  source 1..804: mol_type = other DNA
accgtcttcggtacgcgctcactccgccctctgcctttgttactgccacgtttctctgaatgctctcttgtgtggtgattgctgagagtggtttagctggatctagaattacactctgaaatcgtgttctgcctgtgctgattacttgccgtcctttgtagcagcaaaatatagggacatggtagtacgaaacgaagatagaacctacacagcaatacgagaaatgtgtaatttggtgcttagcggtatttatttaagcacatgttggtgttatagggcacttggattcagaagtttgctgttaatttaggcacaggcttcatactacatgggtcaatagtatagggattcatattataggcgatactataataatttgttcgtctgcagagcttattatttgccaaaattagatattcctattctgtttttgtttgtgtgctgttaaattgttaacgcctgaaggaataaatataaatgacgaaattttgatgtttatctctgctcctttattgtgaccataagtcaagatcagatgcacttgttttaaatattgttgtctgaagaaataagtactgacagtattttgatgcattgatctgcttgtttgttgtaacaaaatttaaaaataaagagtttcctttttgttgctctccttacctcctgatggtatctagtatctaccaactgacactatattgcttctctttacatacgtatcttgctcgatgccttctccctagtgttgaccagtgttactcacatagtctttgctcatttcattgtaatgcagataccaagcgg

SEQ ID NO: 36 - DNA, 228 bp, synthetic construct
  source 1..228: mol_type = other DNA
atggcgcaagttagcaggatctgcaacggcgtgcagaacccgtcgctcatctccaacctctcgaaatccagtcaacgcaaatcgcccttgtcggtgtccctgaagacgcagcagcacccgcgagcctacccgatctcgtcgtcgtggggcttgaagaagagcgggatgacgctgattggctctgagctccgtcccctcaaggtcatgtcttctgtgtccacggcgtgc

SEQ ID NO: 37 - DNA, 505 bp, synthetic construct
  source 1..505: mol_type = other DNA
ctagctatatcatcaatttatgtattacacataatatcgcactcagtctttcatctacggcaatgtaccagctgatataatcagttattgaaatatttctgaatttaaacttgcatcaataaatttatgtttttgcttggactataatacctgacttgttattttatcaataaatatttaaactatatttctttcaagatatcattctttacaagtatacgtgtttaaattgaataccataaatttttatttttcaaatacatgtaaaattatgaaatgggagtggtggcgaccgagctcaagcacacttcaattcctataacggaccaaatcgcaaaaattataataacatattatttcatcctggattaaaagaaagtcaccggggattattttgtgacgccgattacatacggcgacaataaagacattggaaatcgtagtacatattggaatacactgattatattaatgatgaatacatactttaatatccttacgtagg

SEQ ID NO: 38 - DNA, 293 bp, synthetic construct
  source 1..293: mol_type = other DNA
ccgatcctacctgtcacttcatcaaaaggacagtagaaaaggaaggtggcacctacaaatgccatcattgcgataaaggaaaggctatcattcaagatgcctctgccgacagtggtcccaaagatggacccccacccacgaggagcatcgtggaaaaagaagacgttccaaccacgtcttcaaagcaagtggattgatgtgatacttccactgacgtaagggatgacgcacaatcccactatccttcgcaagacccttcctctatataaggaagttcatttcatttggagagg

SEQ ID NO: 39 - DNA, 555 bp, synthetic construct
  source 1..555: mol_type = other DNA
atgtcgcccgagcgcaggcccgtcgagatccgcccggccacagcagccgacatggctgcggtgtgcgacatcgtcaaccactacatcgaaacgtccaccgtgaacttccgcaccgagccgcagacgccgcaggagtggatcgacgaccttgagcgcctccaggaccgctacccctggctcgtcgcggaggtcgaaggcgtcgtggccggcatcgcctacgccgggccgtggaaggctcgcaacgcctacgactggaccgtcgagagcaccgtctacgtgtcccaccgccaccagcgcctgggcctcggctccacgctgtacacgcacctgctcaagtcgatggaggcgcaaggcttcaagagcgtggtcgccgtcatcggcctcccgaacgatccctccgtgaggctccacgaagccctgggctacaccgctcggggcacgctgcgcgcagccggctacaagcacggtggctggcacgacgtcgggttctggcagagggacttcgagctgcccgcgcctccgcgcccggttcgccccgtgacccagatttgatag

SEQ ID NO: 40 - DNA, 175 bp, synthetic construct
  source 1..175: mol_type = other DNA
tttctccataataatgtgtgagtagttcccagataagggaattagggttcctatagggtttcgctcatgtgttgagcatataagaaacccttagtatgtatttgtatttgtaaaatacttctatcaataaaatttctaattcctaaaaccaaaatccagtactaaaatccagatc